European Patent Application EP 4 428 253 A1, published September 11, 2024. Title: Méthode de détermination de la susceptibilité d'une souche de l'espèce Mycobacterium tuberculosis au pyrazinamide. Applicant: BIOMERIEUX. The sequence listing filed with the application follows.

SEQUENCE LISTING (12 sequences)

SEQ ID NO: 1 - DNA, 31 bp, Mycobacterium tuberculosis
  source 1..31: mol_type = genomic DNA
gaccagaacaacccgctgtcggggttgaccc

SEQ ID NO: 2 - DNA, 32 bp, Mycobacterium tuberculosis
  source 1..32: mol_type = genomic DNA
gacagaccgccgggccccagcgccgacagtcg

SEQ ID NO: 3 - DNA, 35 bp, Mycobacterium tuberculosis
  source 1..35: mol_type = genomic DNA
gacccacaagcgccgactgtcggcgctggggcccg

SEQ ID NO: 4 - DNA, 32 bp, Mycobacterium tuberculosis
  source 1..32: mol_type = genomic DNA
ccgacaacctatcgtctcgccgcggccgggcc

SEQ ID NO: 5 - DNA, 40 bp, Mycobacterium tuberculosis
  source 1..40: mol_type = genomic DNA
ggcagtcaccccgacaacctatcgtctcgccgcggccggg

SEQ ID NO: 6 - DNA, 31 bp, Mycobacterium tuberculosis
  source 1..31: mol_type = genomic DNA
accacccgcacggcgacgcgtcgatctacga

SEQ ID NO: 7 - DNA, 49 bp, Mycobacterium tuberculosis
  source 1..49: mol_type = genomic DNA
cggcatcaacggctcgaccacggcccagaactcgtccgaaatcacaccc

SEQ ID NO: 8 - DNA, 32 bp, Mycobacterium tuberculosis
  source 1..32: mol_type = genomic DNA
gcgtcaccggccaatcctcgctggccagtacc

SEQ ID NO: 9 - DNA, 42 bp, Mycobacterium tuberculosis
  source 1..42: mol_type = genomic DNA
cggcgactcgggccatgcccaggatgtagccgtcgtccgacg

SEQ ID NO: 10 - DNA, 33 bp, Mycobacterium tuberculosis
  source 1..33: mol_type = genomic DNA
aacgcggcgtcgatgaggtcgatgtggtcggta

SEQ ID NO: 11 - DNA, 31 bp, Mycobacterium tuberculosis
  source 1..31: mol_type = genomic DNA
cagaagtcgttctgcacgtcgacgatgatca

SEQ ID NO: 12 - DNA, 42 bp, Mycobacterium tuberculosis
  source 1..42: mol_type = genomic DNA
gcaccggaaccggtaaggacgcgatcaccagcggcatcgagg